European Patent Application EP 4 458 355 A1, published November 6, 2024. Title: Taq enzyme reversible modifier, chemically modified Taq enzyme, and preparation method therefor and PCR kit thereof. Applicant: DAAN GENE CO., LTD. The sequence listing filed with the application follows.

SEQUENCE LISTING (2 sequences)

SEQ ID NO: 1 - DNA, 172 bp, synthetic construct
  source 1..172: mol_type = other DNA
gagcccgccgcccggccccgcgcaggccccgcccgggactcccctgcggtccaggccgcgccccgggctccgcgccagccaatgagcgccgcccggccgggcgtgcccccgcgccccaagcataaaccctggcgcgctcgcgggccggcactcttctggtccccacagactc

SEQ ID NO: 2 - DNA, 14 bp, synthetic construct
  source 1..14: mol_type = other DNA
gagtctgtggggag